European Patent Application EP 4 803 629 A1, published September 9, 2026. Title: MULTIVALENT INFLUENZA MRNA VACCINE. Applicant: RINUAGENEBIOTECHNOLOGYCO.,LTD. Application CN. The sequence listing filed with the application follows.

SEQUENCE LISTING (25 sequences)

SEQ ID NO: 1 - DNA, 174 bp, synthetic construct
  source 1..174: mol_type = other DNA; note = nucleotide sequence of the folding region
atgaaggccatcctggtggtgatgctgtacaccttcaccaccgccaacgccgacaccctgtgcatcggctaccacgccaacaacagcaccgacaccgtggacaccgtgctggagaagaacgtgaccgtgacccacagcgtgaacctgctggaggacaagcacaacggcaagctg

SEQ ID NO: 2 - protein, 58 aa, synthetic construct
  source 1..58: note = amino acid sequence of the folding region
MKAILVVMLYTFTTANADTLCIGYHANNSTDTVDTVLEKNVTVTHSVNLLEDKHNGKL

SEQ ID NO: 3 - DNA, 699 bp, synthetic construct
  source 1..699: mol_type = other DNA; note = nucleotide sequence of the HA head of H5N1
tgtgacctggacggcgtgaaacctctgatcctgagagactgcagcgtggccggctggctgctgggcaaccccatgtgcgacgagttcatcaacgtgcccgagtggagctacatcgtggagaaggccaaccccgtgaacgacctgtgctaccccggcgacttcaacgactacgaggagctgaagcacctgctgagcagaatcaaccacttcgagaagattcagatcatccccaagagcagctggagcagccacgaggctagcctgggcgtgagcagcgcctgcccctaccaaggcaagagcagcttcttcagaaacgtggtgtggctgatcaacaagaacagcacctaccccaccatcaagagaagctacaacaacaccaaccaagaggacctgctggtgctgtggggcatccaccaccccaacgacgccgccgagcagaccaagctgtatcagaatcctaccacctacatcagcgtgggcacaagcaccctgaatcagagactggtgcctagaatcgccacaagatccaaggtgaacgggcagagcggcagaatggagttcttctggaccatcctgaagcctaacgacgccatcaacttcgagagcaacggcaacttcatcgcccccgagtacgcctacaagatcgtgaagaagggcgacagcaccatcatgaaaagcgagctggagtacggcaactgc

SEQ ID NO: 4 - protein, 233 aa, synthetic construct
  source 1..233: note = amino acid sequence of the HA head of H5N1
CDLDGVKPLILRDCSVAGWLLGNPMCDEFINVPEWSYIVEKANPVNDLCYPGDFNDYEELKHLLSRINHFEKIQIIPKSSWSSHEASLGVSSACPYQGKSSFFRNVVWLINKNSTYPTIKRSYNNTNQEDLLVLWGIHHPNDAAEQTKLYQNPTTYISVGTSTLNQRLVPRIATRSKVNGQSGRMEFFWTILKPNDAINFESNGNFIAPEYAYKIVKKGDSTIMKSELEYGNC

SEQ ID NO: 5 - DNA, 822 bp, synthetic construct
  source 1..822: mol_type = other DNA; note = nucleotide sequence of the HA stem of H1N1
aacaccacctgtcagacccccgagggcgccatcaacacaagcctgccctttcagaacgtgcaccccatcaccatcggcaagtgccctaagtacgtcaagagcaccaagctgagactggccaccggcctgagaaacgtgcctagcattcagagcagaggcctgttcggcgccatcgccggcttcatcgaaggcggctggaccggcatggtggacggctggtacggctaccaccatcagaacgagcaaggcagcggctacgccgccgatctcaagagcacacagaacgccatcgacaagatcaccaacaaggtgaacagcgtgatcgagaagatgaacacacagttcaccgccgtgggcaaggagttcaaccacctggagaagagaatcgagaacctgaataaaaaggtggacgacggcttcctcgacatctggacctacaacgccgagctgctggtgctgctggagaacgagagaaccctggactaccatgacagcaacgtgaagaacctctacgagaaggtgagaaatcagctgaagaacaacgccaaggagatcggcaacgggtgcttcgagttctaccacaagtgcgacaacacctgcatggagagcgtgaagaacggcacctacgactaccccaagtacagcgaggaggccaagctgaacagagagaagatcgacggcgtgaagctggacagcacaagaatctatcagatcctggccatctacagcaccgtggctagcagcctggtgctcgtggtgagcctgggcgccatcagcttctggatgtgcagcaatggcagcctgcagtgtcggatctgcatc

SEQ ID NO: 6 - protein, 274 aa, synthetic construct
  source 1..274: note = amino acid sequence of the HA stem of H1N1
NTTCQTPEGAINTSLPFQNVHPITIGKCPKYVKSTKLRLATGLRNVPSIQSRGLFGAIAGFIEGGWTGMVDGWYGYHHQNEQGSGYAADLKSTQNAIDKITNKVNSVIEKMNTQFTAVGKEFNHLEKRIENLNKKVDDGFLDIWTYNAELLVLLENERTLDYHDSNVKNLYEKVRNQLKNNAKEIGNGCFEFYHKCDNTCMESVKNGTYDYPKYSEEAKLNREKIDGVKLDSTRIYQILAIYSTVASSLVLVVSLGAISFWMCSNGSLQCRICI

SEQ ID NO: 7 - DNA, 45 bp, synthetic construct
  source 1..45: mol_type = other DNA; note = nucleotide sequence of the flexible linker region
ggcgggggcggctccggcggcgggggcagcggcgggggcggcagc

SEQ ID NO: 8 - protein, 15 aa, synthetic construct
  source 1..15: note = amino acid sequence of the flexible linker region
GGGGSGGGGSGGGGS

SEQ ID NO: 9 - DNA, 1749 bp, synthetic construct
  source 1..1749: mol_type = other DNA; note = nucleotide sequence of the HA coding region of BW
atgaaggctatcatcgtgctgctgatggtggtgacaagcaacgccgacagaatctgcaccggcatcacaagcagcaacagcccccacgtggtgaagaccgccacccaaggcgaggtgaacgtgaccggcgtgatccccctgaccacaacccccaccaagagccacttcgccaacctgaagggcaccgagacaagaggcaagctgtgccccaagtgcctgaactgcaccgacctggacgtggccctgggcagacccaagtgcaccggcaagatccctagcgctagagtgagcatcctgcacgaggtgagacccgtgacaagcggctgcttccccatcatgcacgacagaaccaagatcagacagctgcccaacctgctgagaggctacgagcacgtgagactgagcacccacaacgtgatcaacgccgaggacgcccccggcagaccctacgagatcggcacaagcggcagctgccccaacatcaccaacggcaacggcttcttcgccaccatggcctgggccgtgcccaagaacaaaaccgccaccaaccccctgaccatcgaggtgccctacatctgcaccgagggcgaggatcagatcaccgtgtggggcttccacagcgacagcgagacacagatggccaagctgtacggcgacagcaagcctcagaagttcacaagcagcgccaacggcgtgaccacccactacgtgagccaaatcggcggcttccccaatcagaccgaggacggcggcctgcctcagtccgggagaatcgtggtggactacatggtgcaaaagagcggcaagaccggcaccatcacctatcagagaggcatcctgctgcctcagaaggtgtggtgcgctagcggcagaagcaaggtgattaagggcagcctgcccctgatcggcgaggccgactgcctgcacgagaagtacggcggcctgaacaagagcaagccctactacaccggcgagcacgccaaggccatcggcaactgccccatctgggtgaagacccccctgaagctggccaacggcaccaagtacagaccccccgccaagctgctgaaggagagaggcttcttcggcgccattgccggcttcctggagggcggctgggagggcatgatcgctggctggcacggctatacaagccacggcgctcacggcgtggctgtggctgccgacctcaagagcacccaagaggctatcaacaagattaccaaaaacctgaactccctgagcgagctcgaggtcaagaacctgcagagactgagcggcgccatggacgagctgcacaacgagatcctggagctggacgagaaggtggatgacctgagagccgacaccatcagcagccaaatcgagctggccgtgctgctgagcaacgagggcatcatcaacagcgaggacgagcacctgctggccctggagagaaagctgaagaagatgctgggccctagcgccgtggagattggcaacggctgtttcgagaccaagcacaagtgcaatcagacctgcctggacagaatcgccgccggcaccttcgacgccggcgagttcagcctgcccaccttcgacagcctgaacatcaccgccgctagcctgaacgacgacggcctggacaaccacaccatcctgctgtactacagcacagccgctagctccctggccgtgaccctgatgatcgccatcttcgtggtgtacatggtgagcagagacaacgtgagctgcagcatctgcctgtga

SEQ ID NO: 10 - protein, 582 aa, synthetic construct
  source 1..582: note = amino acid sequence of the HA coding region of BW
MKAIIVLLMVVTSNADRICTGITSSNSPHVVKTATQGEVNVTGVIPLTTTPTKSHFANLKGTETRGKLCPKCLNCTDLDVALGRPKCTGKIPSARVSILHEVRPVTSGCFPIMHDRTKIRQLPNLLRGYEHVRLSTHNVINAEDAPGRPYEIGTSGSCPNITNGNGFFATMAWAVPKNKTATNPLTIEVPYICTEGEDQITVWGFHSDSETQMAKLYGDSKPQKFTSSANGVTTHYVSQIGGFPNQTEDGGLPQSGRIVVDYMVQKSGKTGTITYQRGILLPQKVWCASGRSKVIKGSLPLIGEADCLHEKYGGLNKSKPYYTGEHAKAIGNCPIWVKTPLKLANGTKYRPPAKLLKERGFFGAIAGFLEGGWEGMIAGWHGYTSHGAHGVAVAADLKSTQEAINKITKNLNSLSELEVKNLQRLSGAMDELHNEILELDEKVDDLRADTISSQIELAVLLSNEGIINSEDEHLLALERKLKKMLGPSAVEIGNGCFETKHKCNQTCLDRIAAGTFDAGEFSLPTFDSLNITAASLNDDGLDNHTILLYYSTAASSLAVTLMIAIFVVYMVSRDNVSCSICL

SEQ ID NO: 11 - DNA, 3489 bp, synthetic construct
  source 1..3489: mol_type = other DNA; note = nucleotide sequence of 51-BW
atgaaggccatcctggtggtgatgctgtacaccttcaccaccgccaacgccgacaccctgtgcatcggctaccacgccaacaacagcaccgacaccgtggacaccgtgctggagaagaacgtgaccgtgacccacagcgtgaacctgctggaggacaagcacaacggcaagctgtgtgacctggacggcgtgaaacctctgatcctgagagactgcagcgtggccggctggctgctgggcaaccccatgtgcgacgagttcatcaacgtgcccgagtggagctacatcgtggagaaggccaaccccgtgaacgacctgtgctaccccggcgacttcaacgactacgaggagctgaagcacctgctgagcagaatcaaccacttcgagaagattcagatcatccccaagagcagctggagcagccacgaggctagcctgggcgtgagcagcgcctgcccctaccaaggcaagagcagcttcttcagaaacgtggtgtggctgatcaacaagaacagcacctaccccaccatcaagagaagctacaacaacaccaaccaagaggacctgctggtgctgtggggcatccaccaccccaacgacgccgccgagcagaccaagctgtatcagaatcctaccacctacatcagcgtgggcacaagcaccctgaatcagagactggtgcctagaatcgccacaagatccaaggtgaacgggcagagcggcagaatggagttcttctggaccatcctgaagcctaacgacgccatcaacttcgagagcaacggcaacttcatcgcccccgagtacgcctacaagatcgtgaagaagggcgacagcaccatcatgaaaagcgagctggagtacggcaactgcaacaccacctgtcagacccccgagggcgccatcaacacaagcctgccctttcagaacgtgcaccccatcaccatcggcaagtgccctaagtacgtcaagagcaccaagctgagactggccaccggcctgagaaacgtgcctagcattcagagcagaggcctgttcggcgccatcgccggcttcatcgaaggcggctggaccggcatggtggacggctggtacggctaccaccatcagaacgagcaaggcagcggctacgccgccgatctcaagagcacacagaacgccatcgacaagatcaccaacaaggtgaacagcgtgatcgagaagatgaacacacagttcaccgccgtgggcaaggagttcaaccacctggagaagagaatcgagaacctgaataaaaaggtggacgacggcttcctcgacatctggacctacaacgccgagctgctggtgctgctggagaacgagagaaccctggactaccatgacagcaacgtgaagaacctctacgagaaggtgagaaatcagctgaagaacaacgccaaggagatcggcaacgggtgcttcgagttctaccacaagtgcgacaacacctgcatggagagcgtgaagaacggcacctacgactaccccaagtacagcgaggaggccaagctgaacagagagaagatcgacggcgtgaagctggacagcacaagaatctatcagatcctggccatctacagcaccgtggctagcagcctggtgctcgtggtgagcctgggcgccatcagcttctggatgtgcagcaatggcagcctgcagtgtcggatctgcatcggcgggggcggctccggcggcgggggcagcggcgggggcggcagcatgaaggctatcatcgtgctgctgatggtggtgacaagcaacgccgacagaatctgcaccggcatcacaagcagcaacagcccccacgtggtgaagaccgccacccaaggcgaggtgaacgtgaccggcgtgatccccctgaccacaacccccaccaagagccacttcgccaacctgaagggcaccgagacaagaggcaagctgtgccccaagtgcctgaactgcaccgacctggacgtggccctgggcagacccaagtgcaccggcaagatccctagcgctagagtgagcatcctgcacgaggtgagacccgtgacaagcggctgcttccccatcatgcacgacagaaccaagatcagacagctgcccaacctgctgagaggctacgagcacgtgagactgagcacccacaacgtgatcaacgccgaggacgcccccggcagaccctacgagatcggcacaagcggcagctgccccaacatcaccaacggcaacggcttcttcgccaccatggcctgggccgtgcccaagaacaaaaccgccaccaaccccctgaccatcgaggtgccctacatctgcaccgagggcgaggatcagatcaccgtgtggggcttccacagcgacagcgagacacagatggccaagctgtacggcgacagcaagcctcagaagttcacaagcagcgccaacggcgtgaccacccactacgtgagccaaatcggcggcttccccaatcagaccgaggacggcggcctgcctcagtccgggagaatcgtggtggactacatggtgcaaaagagcggcaagaccggcaccatcacctatcagagaggcatcctgctgcctcagaaggtgtggtgcgctagcggcagaagcaaggtgattaagggcagcctgcccctgatcggcgaggccgactgcctgcacgagaagtacggcggcctgaacaagagcaagccctactacaccggcgagcacgccaaggccatcggcaactgccccatctgggtgaagacccccctgaagctggccaacggcaccaagtacagaccccccgccaagctgctgaaggagagaggcttcttcggcgccattgccggcttcctggagggcggctgggagggcatgatcgctggctggcacggctatacaagccacggcgctcacggcgtggctgtggctgccgacctcaagagcacccaagaggctatcaacaagattaccaaaaacctgaactccctgagcgagctcgaggtcaagaacctgcagagactgagcggcgccatggacgagctgcacaacgagatcctggagctggacgagaaggtggatgacctgagagccgacaccatcagcagccaaatcgagctggccgtgctgctgagcaacgagggcatcatcaacagcgaggacgagcacctgctggccctggagagaaagctgaagaagatgctgggccctagcgccgtggagattggcaacggctgtttcgagaccaagcacaagtgcaatcagacctgcctggacagaatcgccgccggcaccttcgacgccggcgagttcagcctgcccaccttcgacagcctgaacatcaccgccgctagcctgaacgacgacggcctggacaaccacaccatcctgctgtactacagcacagccgctagctccctggccgtgaccctgatgatcgccatcttcgtggtgtacatggtgagcagagacaacgtgagctgcagcatctgcctgtga

SEQ ID NO: 12 - protein, 1162 aa, synthetic construct
  source 1..1162: note = amino acid sequence of 51-BW
MKAILVVMLYTFTTANADTLCIGYHANNSTDTVDTVLEKNVTVTHSVNLLEDKHNGKLCDLDGVKPLILRDCSVAGWLLGNPMCDEFINVPEWSYIVEKANPVNDLCYPGDFNDYEELKHLLSRINHFEKIQIIPKSSWSSHEASLGVSSACPYQGKSSFFRNVVWLINKNSTYPTIKRSYNNTNQEDLLVLWGIHHPNDAAEQTKLYQNPTTYISVGTSTLNQRLVPRIATRSKVNGQSGRMEFFWTILKPNDAINFESNGNFIAPEYAYKIVKKGDSTIMKSELEYGNCNTTCQTPEGAINTSLPFQNVHPITIGKCPKYVKSTKLRLATGLRNVPSIQSRGLFGAIAGFIEGGWTGMVDGWYGYHHQNEQGSGYAADLKSTQNAIDKITNKVNSVIEKMNTQFTAVGKEFNHLEKRIENLNKKVDDGFLDIWTYNAELLVLLENERTLDYHDSNVKNLYEKVRNQLKNNAKEIGNGCFEFYHKCDNTCMESVKNGTYDYPKYSEEAKLNREKIDGVKLDSTRIYQILAIYSTVASSLVLVVSLGAISFWMCSNGSLQCRICIGGGGSGGGGSGGGGSMKAIIVLLMVVTSNADRICTGITSSNSPHVVKTATQGEVNVTGVIPLTTTPTKSHFANLKGTETRGKLCPKCLNCTDLDVALGRPKCTGKIPSARVSILHEVRPVTSGCFPIMHDRTKIRQLPNLLRGYEHVRLSTHNVINAEDAPGRPYEIGTSGSCPNITNGNGFFATMAWAVPKNKTATNPLTIEVPYICTEGEDQITVWGFHSDSETQMAKLYGDSKPQKFTSSANGVTTHYVSQIGGFPNQTEDGGLPQSGRIVVDYMVQKSGKTGTITYQRGILLPQKVWCASGRSKVIKGSLPLIGEADCLHEKYGGLNKSKPYYTGEHAKAIGNCPIWVKTPLKLANGTKYRPPAKLLKERGFFGAIAGFLEGGWEGMIAGWHGYTSHGAHGVAVAADLKSTQEAINKITKNLNSLSELEVKNLQRLSGAMDELHNEILELDEKVDDLRADTISSQIELAVLLSNEGIINSEDEHLLALERKLKKMLGPSAVEIGNGCFETKHKCNQTCLDRIAAGTFDAGEFSLPTFDSLNITAASLNDDGLDNHTILLYYSTAASSLAVTLMIAIFVVYMVSRDNVSCSICL

SEQ ID NO: 13 - DNA, 1701 bp, synthetic construct
  source 1..1701: mol_type = other DNA; note = nucleotide sequence of the HA coding region of H3N2
atgaaaacgattattgcgctgagcaacattctgtgcctggtgtttgcgcaaaagattccgggcaacgataacagcaccgcgaccctgtgcctgggccatcatgcggtgccgaacggcaccgtggtgaaaaccattaccaacgatcgcattgaagtgaccaacgcgaccgaactggtgcagaacagcagcattggcgaaatttgcaacagcccgcatcagattctggatggcggcaactgcaccctgattgatgcgctgctgggcgatccgcagtgcgatggctttcagaacaaagaatgggatctgtttgtggaacgcagccgcgcgaacagcagctgctatccgtatgatgtgccggattatgcgagcctgcgcagcctggtggcgagcagcggcaccctggaatttaaaaacgaaagctttaactggaccggcgtgaaacagaacggcacgagcagcgcgtgcattcgcggcagcagtagcagcttttttagccgcctgaactggctgacgagcctgaacaacatttatccggcgcagaacgtgaccatgccgaacaaagaacagtttgataaactgtatatttggggcgtgcatcatccggataccgataaaaatcagtttagcctgtttgcgcagagcagcggccgcattaccgtgagcaccaaacgcagtcagcaagcggtgattccgaacattggcagccgcccgcgcattcgcgatattccgagccgcattagcatttattggaccattgtgaaaccgggcgatattctgctgattaacagcaccggcaacctgattgcgccgcgcggctattttaaaattcgcagcggcaaaagcagcattatgcgcagcgatgcgccgattggcaaatgcaaaagcgaatgcattaccccgaacggcagcattccgaacgataaaccgtttcagaacgtgaaccgcattacctatggcgcgtgcccgcgctatgtgaaacagagcaccctgaaactggcgaccggcatgcgcaacgtgccggaaaaacagacccgcggcatttttggcgcgattgcgggctttattgaaaacggctgggaaggcatggtggatggctggtatggctttcgccatcagaacagcgaaggccgcggccaagcggcggatctgaaaagcacccaagcggcgattgatcagattagcggcaaactgaaccgcctgattggcaaaaccaacgaaaaatttcatcagattgaaaaagaatttagcgaagtggaaggccgcgtgcaagatctggaaaaatatgtggaagataccaaaattgatctgtggagctataacgcggaactgctggtggcgctggaaaatcagcataccattgatctgaccgatagcgaaatgaacaaactgtttgaaaaaaccaaaaaacagctgcgcgaaaacgcggaagatatgggcaacggctgctttaaaatttatcataaatgcgataacgcgtgcattggcagcattcgcaacgaaacctatgatcataacgtgtatcgcgatgaagcgctgaacaaccgctttcagattaaaggcgtggaactgaaaagcggctataaagattggattctgtggattagctttgcgatgagctgctttctgctgtgcattgcgctgttaggctttattatgtgggcgtgtcagaaaggcaacattcgctgcaacatttgcatttaa

SEQ ID NO: 14 - protein, 566 aa, synthetic construct
  source 1..566: note = amino acid sequence of the HA coding region of H3N2
MKTIIALSNILCLVFAQKIPGNDNSTATLCLGHHAVPNGTVVKTITNDRIEVTNATELVQNSSIGEICNSPHQILDGGNCTLIDALLGDPQCDGFQNKEWDLFVERSRANSSCYPYDVPDYASLRSLVASSGTLEFKNESFNWTGVKQNGTSSACIRGSSSSFFSRLNWLTSLNNIYPAQNVTMPNKEQFDKLYIWGVHHPDTDKNQFSLFAQSSGRITVSTKRSQQAVIPNIGSRPRIRDIPSRISIYWTIVKPGDILLINSTGNLIAPRGYFKIRSGKSSIMRSDAPIGKCKSECITPNGSIPNDKPFQNVNRITYGACPRYVKQSTLKLATGMRNVPEKQTRGIFGAIAGFIENGWEGMVDGWYGFRHQNSEGRGQAADLKSTQAAIDQISGKLNRLIGKTNEKFHQIEKEFSEVEGRVQDLEKYVEDTKIDLWSYNAELLVALENQHTIDLTDSEMNKLFEKTKKQLRENAEDMGNGCFKIYHKCDNACIGSIRNETYDHNVYRDEALNNRFQIKGVELKSGYKDWILWISFAMSCFLLCIALLGFIMWACQKGNIRCNICI

SEQ ID NO: 15 - DNA, 1683 bp, synthetic construct
  source 1..1683: mol_type = other DNA; note = nucleotide sequence of the HA coding region of H7N9
atgaacacacagatcctggtgttcgccctggtggtcgtgatccccacaagcgccgacaagatctgcctgggccaccacgccgtgagcaacggcacaagagtgaacaccctgaccgagagaggcgtggaggtggtgaacgccaccgagaccgtggagagaaccaacgtgcctagaatctgcagcaagggcaagagaaccatcgatctgggccaatgcggcctgctgggcaccatcaccggcccccctcagtgcgatcagttcctggagttcagcgccgacctgatcatcgagagaagagagggcagcgacgtgtgctaccccggcaagttcgtgaacgaggaggccctgagacagatcctgagagagagcggcggcatcgacaaggagaccatgggcttcacctacagcggcatcagaaccaacggcgccaccaacgcctgcagaagaagcggcagcagcttctacgccgagatgaagtggctgctgagcaacaccgacaacgccgccttccctcagatgaccaagagctacaagaacacaagaagagaccccgccctgatcgtgtggggcgtgcaccacagcggcagcaccaccgagcagaccaagctgtacggcagcggcagcaagctgatcaccgtgggcagcagcaactatcagcagagcttcgtgcctagccccggcgctagaccccaagtgaacgggcagagcggcagaatcgacttccactggctgatcctggaccccaacgacaccgtgaccttcagcttcaacggcgccttcatcgcccccgacagagctagcttcctgagaggcaagagcatgggcattcagagcggcgtgcaagtggacgccaactgcgagggcgactgctaccacagcggcggcaccatcatcagcaacctgccctttcagaacatcaacagcagagccgtgggcaagtgccctagatacgtgaagcaagagagcctgatgctggccaccggcatgaagaacgtgcccgagctgcccaagggcagaggcctgttcggcgccatcgccggcttcatcgagaacggctgggagggcctgatcgacggctggtacggcttcagacatcagaacgcccaaggcgagggcaccgccgccgactacaagagcacacagagcgccatcgatcagatcaccggcaagctgaacagactgatcgagaagaccaatcagcagttcgagctgatcgacaacgagttcaccgaggtggagaagcagatcggcaacgtgatcaactggacaagagacagcatgaccgaggtgtggagctacaacgccgagctgctggtggccatggagaatcagcacaccatcgacctcacagacagcgagatgaacaagctgtacgagagagtgagaagacagctgagagagaacgccgaggaggacggcaccggctgcttcgagatcttccacaagtgcgacgacaactgcatggctagcatcagaaacaacacctacgaccacagcaagtacagagaggaggccatgcagaacagaattcagatcgaccccgtgaagctgagcagcggctacaaggacgtgatcctgtggttcagcttcggcgctagctgcttcatcctgctggccatcgccatgggcctggtgttcatctgcgtgaagaacggcaacatgagatgcaccatctgcatctga

SEQ ID NO: 16 - protein, 560 aa, synthetic construct
  source 1..560: note = amino acid sequence of the HA coding region of H7N9
MNTQILVFALVVVIPTSADKICLGHHAVSNGTRVNTLTERGVEVVNATETVERTNVPRICSKGKRTIDLGQCGLLGTITGPPQCDQFLEFSADLIIERREGSDVCYPGKFVNEEALRQILRESGGIDKETMGFTYSGIRTNGATNACRRSGSSFYAEMKWLLSNTDNAAFPQMTKSYKNTRRDPALIVWGVHHSGSTTEQTKLYGSGSKLITVGSSNYQQSFVPSPGARPQVNGQSGRIDFHWLILDPNDTVTFSFNGAFIAPDRASFLRGKSMGIQSGVQVDANCEGDCYHSGGTIISNLPFQNINSRAVGKCPRYVKQESLMLATGMKNVPELPKGRGLFGAIAGFIENGWEGLIDGWYGFRHQNAQGEGTAADYKSTQSAIDQITGKLNRLIEKTNQQFELIDNEFTEVEKQIGNVINWTRDSMTEVWSYNAELLVAMENQHTIDLTDSEMNKLYERVRRQLRENAEEDGTGCFEIFHKCDDNCMASIRNNTYDHSKYREEAMQNRIQIDPVKLSSGYKDVILWFSFGASCFILLAIAMGLVFICVKNGNMRCTICI

SEQ ID NO: 17 - DNA, 1755 bp, synthetic construct
  source 1..1755: mol_type = other DNA; note = nucleotide sequence of the HA coding region of BP
atgaaggccatcatcgtgctgctgatggtggtgacaagcaacgccgacagaatctgcaccggcatcacaagcagcaacagcccccacgtggtgaagaccgccacccaaggcgaggtgaacgtgaccggcgtgatccccctgaccacaacccccaccaagagctacttcgccaacctgaagggcacaagaacaagaggcaagctgtgccccgactgcctgaactgcaccgacctggacgtggccctggggagacccatgtgtgtgggcaccacccctagcgccaaggctagcatcctgcacgaggtgagacccgtgacaagcggctgcttccccatcatgcacgacagaaccaagatcagacagctgcccaacctgctgagaggctacgagaagatcagactgtccacacagaacgtgatcgacgctgaaaaggctcccggcggcccctacagactgggcacaagcggcagctgccccaacgccacaagcaagatcggcttcttcgccaccatggcctgggccgtgcccaaggacaactacaagaacgccaccaaccccctgaccgtggaggtgccctacatctgcaccgagggcgaggatcagatcaccgtgtggggcttccacagcgacgacaagacacagatgaaaagcctgtacggcgacagcaaccctcagaagttcacaagcagcgccaacggcgtgaccacccactacgtgagccaaatcggcgacttccccgatcagaccgaggacggcggcctgcctcagagcggcagaatcgtggtggactacatgatgcagaagcccggcaagaccggcaccatcgtgtatcagagaggcgtgctgctgcctcagaaggtgtggtgcgctagcggcagaagcaaggtgatcaagggcagcctgcccctgatcggcgaggccgactgcctgcacgaggagtacggcggcctgaacaagagcaagccctactacaccggcaagcacgccaaggccatcggcaactgccccatctgggtgaagacccccctgaagctggccaacggcaccaagtacagaccccccgccaagctgctgaaggagagaggcttcttcggcgccatcgccggctttctcgaggggggctgggagggcatgatcgccggctggcatggctacacaagccacggcgcccacggggtcgccgtcgccgccgacctcaagagcacccaagaggccatcaacaagatcaccaagaacctgaacagcctgagcgagctggaggtgaagaacctgcagagactgagcggcgccatggacgagctgcacaacgagatcctggagctggacgagaaggtggacgacctgagagccgacaccatcagcagccaaatcgagctggccgtgctgctgagcaacgagggcatcatcaacagcgaggacgagcacctgctggccctggagagaaagctgaagaagatgctgggccctagcgccgtggacatcggcaacggctgcttcgagaccaagcacaagtgcaatcagacctgcctggacagaatcgccgccggcaccttcaacgccggcgagttcagcctgcccaccttcgacagcctgaacatcaccgccgctagcctgaacgacgacggcctggacaaccacaccatcctgctgtactacagcaccgctgctagctccctcgccgtgaccctgatgctggccatcttcatcgtgtacatggtgagcagagacaacgtgagctgcagcatctgcctgtga

SEQ ID NO: 18 - protein, 584 aa, synthetic construct
  source 1..584: note = amino acid sequence of the HA coding region of BP
MKAIIVLLMVVTSNADRICTGITSSNSPHVVKTATQGEVNVTGVIPLTTTPTKSYFANLKGTRTRGKLCPDCLNCTDLDVALGRPMCVGTTPSAKASILHEVRPVTSGCFPIMHDRTKIRQLPNLLRGYEKIRLSTQNVIDAEKAPGGPYRLGTSGSCPNATSKIGFFATMAWAVPKDNYKNATNPLTVEVPYICTEGEDQITVWGFHSDDKTQMKSLYGDSNPQKFTSSANGVTTHYVSQIGDFPDQTEDGGLPQSGRIVVDYMMQKPGKTGTIVYQRGVLLPQKVWCASGRSKVIKGSLPLIGEADCLHEEYGGLNKSKPYYTGKHAKAIGNCPIWVKTPLKLANGTKYRPPAKLLKERGFFGAIAGFLEGGWEGMIAGWHGYTSHGAHGVAVAADLKSTQEAINKITKNLNSLSELEVKNLQRLSGAMDELHNEILELDEKVDDLRADTISSQIELAVLLSNEGIINSEDEHLLALERKLKKMLGPSAVDIGNGCFETKHKCNQTCLDRIAAGTFNAGEFSLPTFDSLNITAASLNDDGLDNHTILLYYSTAASSLAVTLMLAIFIVYMVSRDNVSCSICL

SEQ ID NO: 19 - DNA, 294 bp, synthetic construct
  source 1..294: mol_type = other DNA; note = nucleotide sequence of the M2 protein
atgagcctgctgaccgaagtggaaaccccgacccgcagcgaatgggaatgccgctgcagcggcagcaacgatccgctggtgattgcggcgaacattattggcattctgcatctgattctgtggattaccgatcgcctgttttttaaatgcatttatcgccgctttaaatatggcctgaaacgcggcccgagcaccgaaggcgtgccggaaagcatgcgcgaagaatatcagcaagaacagcagagcgcggtggatgtggatgatggccattttgtgaacattgaactggaataa

SEQ ID NO: 20 - protein, 97 aa, synthetic construct
  source 1..97: note = amino acid sequence of the M2 protein
MSLLTEVETPTRSEWECRCSGSNDPLVIAANIIGILHLILWITDRLFFKCIYRRFKYGLKRGPSTEGVPESMREEYQQEQQSAVDVDDGHFVNIELE

SEQ ID NO: 21 - DNA, 1695 bp, synthetic construct
  source 1..1695: mol_type = other DNA; note = nucleotide sequence of the 51 chimeric antigen protein
atgaaggccatcctggtggtgatgctgtacaccttcaccaccgccaacgccgacaccctgtgcatcggctaccacgccaacaacagcaccgacaccgtggacaccgtgctggagaagaacgtgaccgtgacccacagcgtgaacctgctggaggacaagcacaacggcaagctgtgtgacctggacggcgtgaaacctctgatcctgagagactgcagcgtggccggctggctgctgggcaaccccatgtgcgacgagttcatcaacgtgcccgagtggagctacatcgtggagaaggccaaccccgtgaacgacctgtgctaccccggcgacttcaacgactacgaggagctgaagcacctgctgagcagaatcaaccacttcgagaagattcagatcatccccaagagcagctggagcagccacgaggctagcctgggcgtgagcagcgcctgcccctaccaaggcaagagcagcttcttcagaaacgtggtgtggctgatcaacaagaacagcacctaccccaccatcaagagaagctacaacaacaccaaccaagaggacctgctggtgctgtggggcatccaccaccccaacgacgccgccgagcagaccaagctgtatcagaatcctaccacctacatcagcgtgggcacaagcaccctgaatcagagactggtgcctagaatcgccacaagatccaaggtgaacgggcagagcggcagaatggagttcttctggaccatcctgaagcctaacgacgccatcaacttcgagagcaacggcaacttcatcgcccccgagtacgcctacaagatcgtgaagaagggcgacagcaccatcatgaaaagcgagctggagtacggcaactgcaacaccacctgtcagacccccgagggcgccatcaacacaagcctgccctttcagaacgtgcaccccatcaccatcggcaagtgccctaagtacgtcaagagcaccaagctgagactggccaccggcctgagaaacgtgcctagcattcagagcagaggcctgttcggcgccatcgccggcttcatcgaaggcggctggaccggcatggtggacggctggtacggctaccaccatcagaacgagcaaggcagcggctacgccgccgatctcaagagcacacagaacgccatcgacaagatcaccaacaaggtgaacagcgtgatcgagaagatgaacacacagttcaccgccgtgggcaaggagttcaaccacctggagaagagaatcgagaacctgaataaaaaggtggacgacggcttcctcgacatctggacctacaacgccgagctgctggtgctgctggagaacgagagaaccctggactaccatgacagcaacgtgaagaacctctacgagaaggtgagaaatcagctgaagaacaacgccaaggagatcggcaacgggtgcttcgagttctaccacaagtgcgacaacacctgcatggagagcgtgaagaacggcacctacgactaccccaagtacagcgaggaggccaagctgaacagagagaagatcgacggcgtgaagctggacagcacaagaatctatcagatcctggccatctacagcaccgtggctagcagcctggtgctcgtggtgagcctgggcgccatcagcttctggatgtgcagcaatggcagcctgcagtgtcggatctgcatc

SEQ ID NO: 22 - protein, 565 aa, synthetic construct
  source 1..565: note = amino acid sequence of the 51 chimeric antigen protein
MKAILVVMLYTFTTANADTLCIGYHANNSTDTVDTVLEKNVTVTHSVNLLEDKHNGKLCDLDGVKPLILRDCSVAGWLLGNPMCDEFINVPEWSYIVEKANPVNDLCYPGDFNDYEELKHLLSRINHFEKIQIIPKSSWSSHEASLGVSSACPYQGKSSFFRNVVWLINKNSTYPTIKRSYNNTNQEDLLVLWGIHHPNDAAEQTKLYQNPTTYISVGTSTLNQRLVPRIATRSKVNGQSGRMEFFWTILKPNDAINFESNGNFIAPEYAYKIVKKGDSTIMKSELEYGNCNTTCQTPEGAINTSLPFQNVHPITIGKCPKYVKSTKLRLATGLRNVPSIQSRGLFGAIAGFIEGGWTGMVDGWYGYHHQNEQGSGYAADLKSTQNAIDKITNKVNSVIEKMNTQFTAVGKEFNHLEKRIENLNKKVDDGFLDIWTYNAELLVLLENERTLDYHDSNVKNLYEKVRNQLKNNAKEIGNGCFEFYHKCDNTCMESVKNGTYDYPKYSEEAKLNREKIDGVKLDSTRIYQILAIYSTVASSLVLVVSLGAISFWMCSNGSLQCRICI

SEQ ID NO: 23 - RNA, 37 nt, synthetic construct
  source 1..37: mol_type = other RNA; note; note (original language) = 5'UTR
actcttctggtccccacagactcagagagaacccacc

SEQ ID NO: 24 - RNA, 110 nt, synthetic construct
  source 1..110: mol_type = other RNA; note; note (original language) = 3'UTR
gctggagcctcggtggccatgcttcttgccccttgggcctccccccagcccctcctccccttcctgcacccgtacccccgtggtctttgaataaagtctgagtgggcggc

SEQ ID NO: 25 - RNA, 123 nt, synthetic construct
  source 1..123: mol_type = other RNA; note; note (original language) = Poly A
aaaaaaaaaaaaaaaaaaaaaaaaaaaaaaaaaaaaaaaaaaaaaaaaaaaaaaaaaaaagatatcaaaaaaaaaaaaaaaaaaagaaaaaaaaaaaaaaaaaaagaaaaaaaaaaaaaaaaa